European Patent Specification EP 3 768 830 B1, published January 25, 2023. Title: PeptiCRAd Cancer Therapy. Applicant: Valo Therapeutics Oy. The sequence listing filed with the application follows.

SEQUENCE LISTING (9 sequences)

SEQ ID NO: 1 - protein, 20 aa, Homo sapiens
VFGIELMEVDPIGHLYIFAT

SEQ ID NO: 2 - protein, 20 aa, Homo sapiens
YLAMPFATPMEAELARRSLA

SEQ ID NO: 3 - protein, 20 aa, Homo sapiens
RGPESRLLEFYLAMPFATPM

SEQ ID NO: 4 - protein, 26 aa, Homo sapiens
KKKKKKVFGIELMEVDPIGHLYIFAT

SEQ ID NO: 5 - protein, 26 aa, Homo sapiens
KKKKKKYLAMPFATPMEAELARRSLA

SEQ ID NO: 6 - protein, 26 aa, Homo sapiens
KKKKKKRGPESRLLEFYLAMPFATPM

SEQ ID NO: 7 - protein, 29 aa, Homo sapiens
KKKKKKKKKVFGIELMEVDPIGHLYIFAT

SEQ ID NO: 8 - protein, 29 aa, Homo sapiens
KKKKKKKKKYLAMPFATPMEAELARRSLA

SEQ ID NO: 9 - protein, 29 aa, Homo sapiens
KKKKKKKKKRGPESRLLEFYLAMPFATPM